European Patent Specification EP 3 411 488 B1, published June 10, 2026. Title: COMPOSITIONS AND METHODS FOR TREATING MPS1. Applicant: The Trustees of the University of Pennsylvania. The sequence listing filed with the application follows.

SEQUENCE LISTING (7 sequences)

SEQ ID NO: 1 - DNA, 1971 bp, Homo sapiens
  CDS (1)..(1971)
atgcggcccctgaggcctagagctgctctgctggcactgctggccagtctgctggctgcccctcctgtggcccctgccgaagcccctcacctggtgcatgtggatgccgccagagccctgtggcctctgcggagattctggcggagcaccggcttttgccccccactgcctcacagccaggccgaccagtacgtgctgagctgggaccagcagctgaacctggcctacgtgggcgccgtgccccacagaggcatcaaacaggtgagaacccactggctgctggaactggtgacaacccggggctccaccggcagaggcctgagctacaacttcacccacctggacggctacctggacctgctgagagagaaccagctgctgcccggcttcgagctgatgggcagcgccagcggccacttcaccgacttcgaggacaagcagcaagtctttgagtggaaggacctggtgtccagcctggccagacggtacatcggcagatacggactggcccacgtgtccaagtggaacttcgagacatggaacgagcccgaccaccacgacttcgacaacgtgtcaatgaccatgcagggctttctgaactactacgacgcctgctccgagggcctgagagccgccagtcctgccctgagactgggcggacccggcgatagcttccacaccccccccagaagccccctgagctggggcctgctgagacactgccacgacggcaccaatttcttcaccggcgaggccggcgtgcggctggactacatcagcctgcaccggaagggcgccagaagcagcatcagcatcctggaacaggaaaaggtcgtcgcccagcagatccggcagctgttccccaagttcgccgacacccccatctacaacgacgaggccgaccccctggtgggatggtcactgcctcagccttggagagccgacgtgacctacgccgctatggtggtgaaagtgatcgcccagcatcagaacctgctgctggccaacaccaccagcgccttcccttacgccctgctgagcaacgacaacgccttcctgagctaccacccccaccccttcgcccagagaaccctgaccgcccggttccaggtgaacaacaccagacccccccacgtgcagctgctgagaaagcccgtgctgaccgctatgggactgctggctctgctggacgaggaacagctgtgggccgaagtgtcccaggccggcaccgtgctggacagcaatcatacagtgggcgtgctggcctccgcccacagacctcagggacccgccgatgcttggcgggctgccgtgctgatctacgccagcgacgataccagagcccaccccaacagatccgtggccgtgaccctgcggctgagaggcgtgccaccaggccctggactggtgtacgtgaccagatacctggacaacggcctgtgcagccccgacggcgaatggcgcagactgggcagacctgtgttccccaccgccgagcagttccggcggatgagagccgctgaggatcctgtggctgctgcccctagacctctgcctgctggcggcagactgaccctgaggcccgctctgagactgcctagtctgctgctggtgcacgtgtgcgccaggcccgagaagcctcccggccaggtgacaagactgagagccctgcccctgacccagggccagctggtgctggtgtggtccgatgagcacgtgggcagcaagtgcctgtggacctacgagatccagttcagccaggacggcaaggcctacacccccgtgtcccggaagcccagcaccttcaacctgttcgtgttcagccccgatacaggcgccgtgtccggctcttatagagtgcgggccctggactactgggccagacccggccctttcagcgaccccgtgccctacctggaagtgcccgtgcctagaggcccccctagccccggcaacccttgagtcgacccg

SEQ ID NO: 2 - protein, 653 aa, Homo sapiens
MRPLRPRAALLALLASLLAAPPVAPAEAPHLVHVDAARALWPLRRFWRSTGFCPPLPHSQADQYVLSWDQQLNLAYVGAVPHRGIKQVRTHWLLELVTTRGSTGRGLSYNFTHLDGYLDLLRENQLLPGFELMGSASGHFTDFEDKQQVFEWKDLVSSLARRYIGRYGLAHVSKWNFETWNEPDHHDFDNVSMTMQGFLNYYDACSEGLRAASPALRLGGPGDSFHTPPRSPLSWGLLRHCHDGTNFFTGEAGVRLDYISLHRKGARSSISILEQEKVVAQQIRQLFPKFADTPIYNDEADPLVGWSLPQPWRADVTYAAMVVKVIAQHQNLLLANTTSAFPYALLSNDNAFLSYHPHPFAQRTLTARFQVNNTRPPHVQLLRKPVLTAMGLLALLDEEQLWAEVSQAGTVLDSNHTVGVLASAHRPQGPADAWRAAVLIYASDDTRAHPNRSVAVTLRLRGVPPGPGLVYVTRYLDNGLCSPDGEWRRLGRPVFPTAEQFRRMRAAEDPVAAAPRPLPAGGRLTLRPALRLPSLLLVHVCARPEKPPGQVTRLRALPLTQGQLVLVWSDEHVGSKCLWTYEIQFSQDGKAYTPVSRKPSTFNLFVFSPDTGAVSGSYRVRALDYWARPGPFSDPVPYLEVPVPRGPPSPGNP

SEQ ID NO: 3 - DNA, 4344 bp, Artificial sequence
  CB7.CI.hIDUAco.RBG
  misc_feature (1)..(130): 5"ITR
  promoter (198)..(579): CMV IE promoter
  promoter (582)..(863): CB promoter
  TATA_signal (836)..(839)
  Intron (956)..(1928): chicken beta-actin intron
  CDS (1990)..(3948): human IDUA co
  polyA_signal (4000)..(4126): rabbit globin polyA
  misc_feature (4215)..(4344)
ctgcgcgctcgctcgctcactgaggccgcccgggcaaagcccgggcgtcgggcgacctttggtcgcccggcctcagtgagcgagcgagcgcgcagagagggagtggccaactccatcactaggggttccttgtagttaatgattaacccgccatgctacttatctaccagggtaatggggatcctctagaactatagctagtcgacattgattattgactagttattaatagtaatcaattacggggtcattagttcatagcccatatatggagttccgcgttacataacttacggtaaatggcccgcctggctgaccgcccaacgacccccgcccattgacgtcaataatgacgtatgttcccatagtaacgccaatagggactttccattgacgtcaatgggtggagtatttacggtaaactgcccacttggcagtacatcaagtgtatcatatgccaagtacgccccctattgacgtcaatgacggtaaatggcccgcctggcattatgcccagtacatgaccttatgggactttcctacttggcagtacatctacgtattagtcatcgctattaccatggtcgaggtgagccccacgttctgcttcactctccccatctcccccccctccccacccccaattttgtatttatttattttttaattattttgtgcagcgatgggggcggggggggggggggggcgcgcgccaggcggggcggggcggggcgaggggcggggcggggcgaggcggagaggtgcggcggcagccaatcagagcggcgcgctccgaaagtttccttttatggcgaggcggcggcggcggcggccctataaaaagcgaagcgcgcggcgggcgggagtcgctgcgcgctgccttcgccccgtgccccgctccgccgccgcctcgcgccgcccgccccggctctgactgaccgcgttactcccacaggtgagcgggcgggacggcccttctcctccgggctgtaattagcgcttggtttaatgacggcttgtttcttttctgtggctgcgtgaaagccttgaggggctccgggagggccctttgtgcggggggagcggctcggggggtgcgtgcgtgtgtgtgtgcgtggggagcgccgcgtgcggctccgcgctgcccggcggctgtgagcgctgcgggcgcggcgcggggctttgtgcgctccgcagtgtgcgcgaggggagcgcggccgggggcggtgccccgcggtgcggggggggctgcgaggggaacaaaggctgcgtgcggggtgtgtgcgtgggggggtgagcagggggtgtgggcgcgtcggtcgggctgcaaccccccctgcacccccctccccgagttgctgagcacggcccggcttcgggtgcggggctccgtacggggcgtggcgcggggctcgccgtgccgggcggggggtggcggcaggtgggggtgccgggcggggcggggccgcctcgggccggggagggctcgggggaggggcgcggcggcccccggagcgccggcggctgtcgaggcgcggcgagccgcagccattgccttttatggtaatcgtgcgagagggcgcagggacttcctttgtcccaaatctgtgcggagccgaaatctgggaggcgccgccgcaccccctctagcgggcgcggggcgaagcggtgcggcgccggcaggaaggaaatgggcggggagggccttcgtgcgtcgccgcgccgccgtccccttctccctctccagcctcggggctgtccgcggggggacggctgccttcgggggggacggggcagggcggggttcggcttctggcgtgtgaccggcggctctagagcctctgctaaccatgttcatgccttcttctttttcctacagctcctgggcaacgtgctggttattgtgctgtctcatcattttggcaaagaattcacgcgtggtacctctagagtcgacccgggcggcctcgagaattcacgcgtgccaccatgcggcccctgaggcctagagctgctctgctggcactgctggccagtctgctggctgcccctcctgtggcccctgccgaagcccctcacctggtgcatgtggatgccgccagagccctgtggcctctgcggagattctggcggagcaccggcttttgccccccactgcctcacagccaggccgaccagtacgtgctgagctgggaccagcagctgaacctggcctacgtgggcgccgtgccccacagaggcatcaaacaggtgagaacccactggctgctggaactggtgacaacccggggctccaccggcagaggcctgagctacaacttcacccacctggacggctacctggacctgctgagagagaaccagctgctgcccggcttcgagctgatgggcagcgccagcggccacttcaccgacttcgaggacaagcagcaagtctttgagtggaaggacctggtgtccagcctggccagacggtacatcggcagatacggactggcccacgtgtccaagtggaacttcgagacatggaacgagcccgaccaccacgacttcgacaacgtgtcaatgaccatgcagggctttctgaactactacgacgcctgctccgagggcctgagagccgccagtcctgccctgagactgggcggacccggcgatagcttccacaccccccccagaagccccctgagctggggcctgctgagacactgccacgacggcaccaatttcttcaccggcgaggccggcgtgcggctggactacatcagcctgcaccggaagggcgccagaagcagcatcagcatcctggaacaggaaaaggtcgtcgcccagcagatccggcagctgttccccaagttcgccgacacccccatctacaacgacgaggccgaccccctggtgggatggtcactgcctcagccttggagagccgacgtgacctacgccgctatggtggtgaaagtgatcgcccagcatcagaacctgctgctggccaacaccaccagcgccttcccttacgccctgctgagcaacgacaacgccttcctgagctaccacccccaccccttcgcccagagaaccctgaccgcccggttccaggtgaacaacaccagacccccccacgtgcagctgctgagaaagcccgtgctgaccgctatgggactgctggctctgctggacgaggaacagctgtgggccgaagtgtcccaggccggcaccgtgctggacagcaatcatacagtgggcgtgctggcctccgcccacagacctcagggacccgccgatgcttggcgggctgccgtgctgatctacgccagcgacgataccagagcccaccccaacagatccgtggccgtgaccctgcggctgagaggcgtgccaccaggccctggactggtgtacgtgaccagatacctggacaacggcctgtgcagccccgacggcgaatggcgcagactgggcagacctgtgttccccaccgccgagcagttccggcggatgagagccgctgaggatcctgtggctgctgcccctagacctctgcctgctggcggcagactgaccctgaggcccgctctgagactgcctagtctgctgctggtgcacgtgtgcgccaggcccgagaagcctcccggccaggtgacaagactgagagccctgcccctgacccagggccagctggtgctggtgtggtccgatgagcacgtgggcagcaagtgcctgtggacctacgagatccagttcagccaggacggcaaggcctacacccccgtgtcccggaagcccagcaccttcaacctgttcgtgttcagccccgatacaggcgccgtgtccggctcttatagagtgcgggccctggactactgggccagacccggccctttcagcgaccccgtgccctacctggaagtgcccgtgcctagaggcccccctagccccggcaacccttgagtcgacccgggcggcctcgaggacggggtgaactacgcctgaggatccgatctttttccctctgccaaaaattatggggacatcatgaagccccttgagcatctgacttctggctaataaaggaaatttattttcattgcaatagtgtgttggaattttttgtgtctctcactcggaagcaattcgttgatctgaatttcgaccacccataatacccattaccctggtagataagtagcatggcgggttaatcattaactacaaggaacccctagtgatggagttggccactccctctctgcgcgctcgctcgctcactgaggccgggcgaccaaaggtcgcccgacgcccgggctttgcccgggcggcctcagtgagcgagcgagcgcgcag

SEQ ID NO: 4 - protein, 653 aa, Artificial sequence; identical to SEQ ID NO: 2
  Synthetic Construct

SEQ ID NO: 5 - DNA, 3605 bp, Artificial sequence
  Vector genome - TBG.PI.hIDUAco.RBG
  repeat_region (1)..(130): 5' ITR
  enhancer (221)..(320): Alpha mic/Bik
  enhancer (327)..(426): Alpha mic/Bik
  promoter (442)..(901): TBG
  TATA_signal (885)..(888)
  Intron (1027)..(1157)
  misc_feature (1251)..(3212): Human alpha-L-IDUA coding sequence
  polyA_signal (3261)..(3387): rabbit globin poly A
  repeat_region (3476)..(3605)
ctgcgcgctcgctcgctcactgaggccgcccgggcaaagcccgggcgtcgggcgacctttggtcgcccggcctcagtgagcgagcgagcgcgcagagagggagtggccaactccatcactaggggttccttgtagttaatgattaacccgccatgctacttatctaccagggtaatggggatcctctagaactatagctagaattcgcccttaagctagcaggttaatttttaaaaagcagtcaaaagtccaagtggcccttggcagcatttactctctctgtttgctctggttaataatctcaggagcacaaacattccagatccaggttaatttttaaaaagcagtcaaaagtccaagtggcccttggcagcatttactctctctgtttgctctggttaataatctcaggagcacaaacattccagatccggcgcgccagggctggaagctacctttgacatcatttcctctgcgaatgcatgtataatttctacagaacctattagaaaggatcacccagcctctgcttttgtacaactttcccttaaaaaactgccaattccactgctgtttggcccaatagtgagaactttttcctgctgcctcttggtgcttttgcctatggcccctattctgcctgctgaagacactcttgccagcatggacttaaacccctccagctctgacaatcctctttctcttttgttttacatgaagggtctggcagccaaagcaatcactcaaagttcaaaccttatcattttttgctttgttcctcttggccttggttttgtacatcagctttgaaaataccatcccagggttaatgctggggttaatttataactaagagtgctctagttttgcaatacaggacatgctataaaaatggaaagatgttgctttctgagagacagctttattgcggtagtttatcacagttaaattgctaacgcagtcagtgcttctgacacaacagtctcgaacttaagctgcagaagttggtcgtgaggcactgggcaggtaagtatcaaggttacaagacaggtttaaggagaccaatagaaactgggcttgtcgagacagagaagactcttgcgtttctgataggcacctattggtcttactgacatccactttgcctttctctccacaggtgtccactcccagttcaattacagctcttaaggctagagtacttaatacgactcactataggctagcctcgagaattcacgcgtgccaccatgcggcccctgaggcctagagctgctctgctggcactgctggccagtctgctggctgcccctcctgtggcccctgccgaagcccctcacctggtgcatgtggatgccgccagagccctgtggcctctgcggagattctggcggagcaccggcttttgccccccactgcctcacagccaggccgaccagtacgtgctgagctgggaccagcagctgaacctggcctacgtgggcgccgtgccccacagaggcatcaaacaggtgagaacccactggctgctggaactggtgacaacccggggctccaccggcagaggcctgagctacaacttcacccacctggacggctacctggacctgctgagagagaaccagctgctgcccggcttcgagctgatgggcagcgccagcggccacttcaccgacttcgaggacaagcagcaagtctttgagtggaaggacctggtgtccagcctggccagacggtacatcggcagatacggactggcccacgtgtccaagtggaacttcgagacatggaacgagcccgaccaccacgacttcgacaacgtgtcaatgaccatgcagggctttctgaactactacgacgcctgctccgagggcctgagagccgccagtcctgccctgagactgggcggacccggcgatagcttccacaccccccccagaagccccctgagctggggcctgctgagacactgccacgacggcaccaatttcttcaccggcgaggccggcgtgcggctggactacatcagcctgcaccggaagggcgccagaagcagcatcagcatcctggaacaggaaaaggtcgtcgcccagcagatccggcagctgttccccaagttcgccgacacccccatctacaacgacgaggccgaccccctggtgggatggtcactgcctcagccttggagagccgacgtgacctacgccgctatggtggtgaaagtgatcgcccagcatcagaacctgctgctggccaacaccaccagcgccttcccttacgccctgctgagcaacgacaacgccttcctgagctaccacccccaccccttcgcccagagaaccctgaccgcccggttccaggtgaacaacaccagacccccccacgtgcagctgctgagaaagcccgtgctgaccgctatgggactgctggctctgctggacgaggaacagctgtgggccgaagtgtcccaggccggcaccgtgctggacagcaatcatacagtgggcgtgctggcctccgcccacagacctcagggacccgccgatgcttggcgggctgccgtgctgatctacgccagcgacgataccagagcccaccccaacagatccgtggccgtgaccctgcggctgagaggcgtgccaccaggccctggactggtgtacgtgaccagatacctggacaacggcctgtgcagccccgacggcgaatggcgcagactgggcagacctgtgttccccaccgccgagcagttccggcggatgagagccgctgaggatcctgtggctgctgcccctagacctctgcctgctggcggcagactgaccctgaggcccgctctgagactgcctagtctgctgctggtgcacgtgtgcgccaggcccgagaagcctcccggccaggtgacaagactgagagccctgcccctgacccagggccagctggtgctggtgtggtccgatgagcacgtgggcagcaagtgcctgtggacctacgagatccagttcagccaggacggcaaggcctacacccccgtgtcccggaagcccagcaccttcaacctgttcgtgttcagccccgatacaggcgccgtgtccggctcttatagagtgcgggccctggactactgggccagacccggccctttcagcgaccccgtgccctacctggaagtgcccgtgcctagaggcccccctagccccggcaacccttgagtcgacccgggcggcctcgaggacggggtgaactacgcctgaggatccgatctttttccctctgccaaaaattatggggacatcatgaagccccttgagcatctgacttctggctaataaaggaaatttattttcattgcaatagtgtgttggaattttttgtgtctctcactcggaagcaattcgttgatctgaatttcgaccacccataatacccattaccctggtagataagtagcatggcgggttaatcattaactacaaggaacccctagtgatggagttggccactccctctctgcgcgctcgctcgctcactgaggccgggcgaccaaaggtcgcccgacgcccgggctttgcccgggcggcctcagtgagcgagcgagcgcgcag

SEQ ID NO: 6 - DNA, 3691 bp, Artificial sequence
  Vector genome: CMV.PI.hIDUAco.SV40
  repeat_region (1)..(130): 5' ITR
  misc_feature (143)..(181): CMV enhancer and promoter
  TATA_signal (910)..(916)
  Intron (1024)..(1221): chimeric intron
  misc_feature (1284)..(3246): human IDUA coding sequence
  polyA_signal (3258)..(3496)
  repeat_region (3562)..(3691)
ggccttaattaggctgcgcgctcgctcgctcactgaggccgcccgggcaaagcccgggcgtcgggcgacctttggtcgcccggcctcagtgagcgagcgagcgcgcagagagggagtggccaactccatcactaggggttccttgtagttaatgattaacccgccatgctacttatctacgtagccatgctctaggaagatcttcaatattggccattagccatattattcattggttatatagcataaatcaatattggctattggccattgcatacgttgtatctatatcataatatgtacatttatattggctcatgtccaatatgaccgccatgttggcattgattattgactagttattaatagtaatcaattacggggtcattagttcatagcccatatatggagttccgcgttacataacttacggtaaatggcccgcctggctgaccgcccaacgacccccgcccattgacgtcaataatgacgtatgttcccatagtaacgccaatagggactttccattgacgtcaatgggtggagtatttacggtaaactgcccacttggcagtacatcaagtgtatcatatgccaagtccgccccctattgacgtcaatgacggtaaatggcccgcctggcattatgcccagtacatgaccttacgggactttcctacttggcagtacatctacgtattagtcatcgctattaccatggtgatgcggttttggcagtacaccaatgggcgtggatagcggtttgactcacggggatttccaagtctccaccccattgacgtcaatgggagtttgttttggcaccaaaatcaacgggactttccaaaatgtcgtaataaccccgccccgttgacgcaaatgggcggtaggcgtgtacggtgggaggtctatataagcagagctcgtttagtgaaccgtcagatcactagaagctttattgcggtagtttatcacagttaaattgctaacgcagtcagtgcttctgacacaacagtctcgaacttaagctgcagaagttggtcgtgaggcactgggcaggtaagtatcaaggttacaagacaggtttaaggagaccaatagaaactgggcttgtcgagacagagaagactcttgcgtttctgataggcacctattggtcttactgacatccactttgcctttctctccacaggtgtccactcccagttcaattacagctcttaaggctagagtacttaatacgactcactataggctagcctcgagaattcacgcgtgccaccatgcggcccctgaggcctagagctgctctgctggcactgctggccagtctgctggctgcccctcctgtggcccctgccgaagcccctcacctggtgcatgtggatgccgccagagccctgtggcctctgcggagattctggcggagcaccggcttttgccccccactgcctcacagccaggccgaccagtacgtgctgagctgggaccagcagctgaacctggcctacgtgggcgccgtgccccacagaggcatcaaacaggtgagaacccactggctgctggaactggtgacaacccggggctccaccggcagaggcctgagctacaacttcacccacctggacggctacctggacctgctgagagagaaccagctgctgcccggcttcgagctgatgggcagcgccagcggccacttcaccgacttcgaggacaagcagcaagtctttgagtggaaggacctggtgtccagcctggccagacggtacatcggcagatacggactggcccacgtgtccaagtggaacttcgagacatggaacgagcccgaccaccacgacttcgacaacgtgtcaatgaccatgcagggctttctgaactactacgacgcctgctccgagggcctgagagccgccagtcctgccctgagactgggcggacccggcgatagcttccacaccccccccagaagccccctgagctggggcctgctgagacactgccacgacggcaccaatttcttcaccggcgaggccggcgtgcggctggactacatcagcctgcaccggaagggcgccagaagcagcatcagcatcctggaacaggaaaaggtcgtcgcccagcagatccggcagctgttccccaagttcgccgacacccccatctacaacgacgaggccgaccccctggtgggatggtcactgcctcagccttggagagccgacgtgacctacgccgctatggtggtgaaagtgatcgcccagcatcagaacctgctgctggccaacaccaccagcgccttcccttacgccctgctgagcaacgacaacgccttcctgagctaccacccccaccccttcgcccagagaaccctgaccgcccggttccaggtgaacaacaccagacccccccacgtgcagctgctgagaaagcccgtgctgaccgctatgggactgctggctctgctggacgaggaacagctgtgggccgaagtgtcccaggccggcaccgtgctggacagcaatcatacagtgggcgtgctggcctccgcccacagacctcagggacccgccgatgcttggcgggctgccgtgctgatctacgccagcgacgataccagagcccaccccaacagatccgtggccgtgaccctgcggctgagaggcgtgccaccaggccctggactggtgtacgtgaccagatacctggacaacggcctgtgcagccccgacggcgaatggcgcagactgggcagacctgtgttccccaccgccgagcagttccggcggatgagagccgctgaggatcctgtggctgctgcccctagacctctgcctgctggcggcagactgaccctgaggcccgctctgagactgcctagtctgctgctggtgcacgtgtgcgccaggcccgagaagcctcccggccaggtgacaagactgagagccctgcccctgacccagggccagctggtgctggtgtggtccgatgagcacgtgggcagcaagtgcctgtggacctacgagatccagttcagccaggacggcaaggcctacacccccgtgtcccggaagcccagcaccttcaacctgttcgtgttcagccccgatacaggcgccgtgtccggctcttatagagtgcgggccctggactactgggccagacccggccctttcagcgaccccgtgccctacctggaagtgcccgtgcctagaggcccccctagccccggcaacccttgagtcgacccgggcggccgcttcgagcagacatgataagatacattgatgagtttggacaaaccacaactagaatgcagtgaaaaaaatgctttatttgtgaaatttgtgatgctattgctttatttgtaaccattataagctgcaataaacaagttaacaacaacaattgcattcattttatgtttcaggttcagggggagatgtgggaggttttttaaagcaagtaaaacctctacaaatgtggtaaaatcgataaggatcttcctagagcatggctacgtagataagtagcatggcgggttaatcattaactacaaggaacccctagtgatggagttggccactccctctctgcgcgctcgctcgctcactgaggccgggcgaccaaaggtcgcccgacgcccgggctttgcccgggcggcctcagtgagcgagcgagcgcgcag

SEQ ID NO: 7 - protein, 736 aa, Artificial sequence
  hu14/Adeno-associated virus 9
MAADGYLPDWLEDNLSEGIREWWALKPGAPQPKANQQHQDNARGLVLPGYKYLGPGNGLDKGEPVNAADAAALEHDKAYDQQLKAGDNPYLKYNHADAEFQERLKEDTSFGGNLGRAVFQAKKRLLEPLGLVEEAAKTAPGKKRPVEQSPQEPDSSAGIGKSGAQPAKKRLNFGQTGDTESVPDPQPIGEPPAAPSGVGSLTMASGGGAPVADNNEGADGVGSSSGNWHCDSQWLGDRVITTSTRTWALPTYNNHLYKQISNSTSGGSSNDNAYFGYSTPWGYFDFNRFHCHFSPRDWQRLINNNWGFRPKRLNFKLFNIQVKEVTDNNGVKTIANNLTSTVQVFTDSDYQLPYVLGSAHEGCLPPFPADVFMIPQYGYLTLNDGSQAVGRSSFYCLEYFPSQMLRTGNNFQFSYEFENVPFHSSYAHSQSLDRLMNPLIDQYLYYLSKTINGSGQNQQTLKFSVAGPSNMAVQGRNYIPGPSYRQQRVSTTVTQNNNSEFAWPGASSWALNGRNSLMNPGPAMASHKEGEDRFFPLSGSLIFGKQGTGRDNVDADKVMITNEEEIKTTNPVATESYGQVATNHQSAQAQAQTGWVQNQGILPGMVWQDRDVYLQGPIWAKIPHTDGNFHPSPLMGGFGMKHPPPQILIKNTPVPADPPTAFNKDKLNSFITQYSTGQVSVEIEWELQKENSKRWNPEIQYTSNYYKSNNVEFAVNTEGVYSEPRPIGTRYLTRNL